European Patent Application EP 4 375 296 A1, published May 29, 2024. Title: AN A-FABP NEUTRALIZING MONOCLONAL ANTIBODY AND PREPARATION METHOD AND USE THEREOF. Applicant: Versitech Limited. The sequence listing filed with the application follows.

SEQUENCE LISTING (11 sequences)

SEQ ID NO: 1 - protein, 5 aa, synthetic construct
DYNMD

SEQ ID NO: 2 - protein, 17 aa, synthetic construct
DINPYNGDTIYNQNFKG

SEQ ID NO: 3 - protein, 4 aa, synthetic construct
GYGF

SEQ ID NO: 4 - protein, 16 aa, synthetic construct
RSSQSLVYINGNTYLH

SEQ ID NO: 5 - protein, 7 aa, synthetic construct
KVSNRFS

SEQ ID NO: 6 - protein, 9 aa, synthetic construct
SQSTHVPYT

SEQ ID NO: 7 - protein, 112 aa, synthetic construct
VKLQESGPELVKPGASVKIPCKASGYTFTDYNMDWVRQSRGKSLEWIGDINPYNGDTIYNQNFKGKATLTVDKSSTTAYLELRSLTSEDTAVYYCASGYGFWGQGTTVTVSS

SEQ ID NO: 8 - protein, 112 aa, synthetic construct
DIVMTQAPLSLPVSLGAQASISCRSSQSLVYINGNTYLHWYLQKPGQSPKLLIYKVSNRFSGVPDRFSGSGSGTDFTLKISRVEAEDLGVYFCSQSTHVPYTFGGGTKLEIK

SEQ ID NO: 9 - protein, 636 aa, synthetic construct
VKLQESGPELVKPGASVKIPCKASGYTFTDYNMDWVRQSRGKSLEWIGDINPYNGDTIYNQNFKGKATLTVDKSSTTAYLELRSLTSEDTAVYYCASGYGFWGQGTTVTVSSASTKGPSVFPLAPCSRSTSESTAALGCLVKDYFPEPVTVSWNSGALTSGVHTFPAVLQSSGLYSLSSVVTVPSSSLGTKTYTCNVDHKPSNTKVDKRVESKYGPPCPSCPAPEFLGGPSVFLFPPKPKDTLMISRTPEVTCVVVDVSQEDPEVQFNWYVDGVEVHNAKTKPREEQFNSTYRVVSVLTVLHQDWLNGKEYKCKVSNKGLPSSIEKTISKAKPSVFLFPPKPKDTLMISRTPEVTCVVVDVSQEDPEVQFNWYVDGVEVHNAKTKPREEQFNSTYRVVSVLTVLHQDWLNGKEYKCKVSNKGLPSSIEKTISGQPREPQVYTLPPSQEEMTKNQVSLTCLVKGFYPSDIAVEWESNGQPENNYKTTPPVLDSDGSFFLYSRLTVDKSRWQEGNVFSCSVMHEALHNHYTQKSLSLSLGKPQVYTLPPSQEEMTKNQVSLTCLVKGFYPSDIAVEWESNGQPENNYKTTPPVLDSDGSFFLYSRLTVDKSRWQEGNVFSCSVMHEALHNHYTQKSLS

SEQ ID NO: 10 - protein, 207 aa, synthetic construct
DIVMTQAPLSLPVSLGAQASISCRSSQSLVYINGNTYLHWYLQKPGQSPKLLIYKVSNRFSGVPDRFSGSGSGTDFTLKISRVEAEDLGVYFCSQSTHVPYTFGGGTKLEIKPTVTLFPPSSEELQANKATLVCLISDFYPGAVTVAWKADGSPVKAGVETTKPSKQSNNKYAASSYLSLTPEQWKSHRSYSCQVTHEGSTVEKTVA

SEQ ID NO: 11 - protein, 15 aa, synthetic construct
KEVGVGFATRKVAGC